European Patent Application EP 4 375 379 A1, published May 29, 2024. Title: BIOPRODUCTION OF GLYCOLIC ACID FROM GLYOXAL. Applicant: BIOC3. The sequence listing filed with the application follows.

SEQUENCE LISTING (8 sequences)

SEQ ID NO: 1 - protein, 172 aa, Escherichia coli
MSKKIAVLITDEFEDSEFTSPADEFRKAGHEVITIEKQAGKTVKGKKGEASVTIDKSIDEVTPAEFDALLLPGGHSPDYLRGDNRFVTFTRDFVNSGKPVFAICHGPQLLISADVIRGRKLTAVKPIIIDVKNAGAEFYDQEVVVDKDQLVTSRTPDDLPAFNREALRLLGA

SEQ ID NO: 2 - DNA, 519 bp, Escherichia coli
  source 1..519: mol_type = genomic DNA
atgagtaagaaaattgccgttttaatcactgatgaatttgaggattcagaatttacttcacccgcagacgagttccgtaaagccggacacgaagtgattaccattgaaaaacaagcgggtaaaacggtgaaaggcaaaaaaggagaagccagcgtgaccatcgataaatccatcgatgaagtgacgcctgcggagtttgatgccctgctgctaccgggcggccattcaccggattatctgcgtggggacaaccgttttgtcacctttacccgtgattttgtgaatagtggcaaaccggtgtttgccatctgtcacggcccgcagttgctgatcagcgccgatgtgattcgggggcgcaaactgaccgcagttaaaccgatcattattgatgttaaaaatgcgggcgcggaattttacgatcaggaagtcgtggttgataaagatcagctggttaccagccggacaccggacgatctgccagcgtttaaccgcgaggcgttacgcctgctcggtgcctga

SEQ ID NO: 3 - protein, 169 aa, Escherichia coli
KKIAVLITDEFEDSEFTSPADEFRKAGHEVITIEKQAGKTVKGKKGEASVTIDKSIDEVTPAEFDALLLPGGHSPDYLRGDNRFVTFTRDFVNSGKPVFAICHGPQLLISADVIRGRKLTAVKPIIIDVKNAGAEFYDQEVVVDKDQLVTSRTPDDLPAFNREALRLLG

SEQ ID NO: 4 - DNA, 510 bp, Escherichia coli
  source 1..510: mol_type = genomic DNA
aagaaaattgccgttttaatcactgatgaatttgaggattcagaatttacttcacccgcagacgagttccgtaaagccggacacgaagtgattaccattgaaaaacaagcgggtaaaacggtgaaaggcaaaaaaggagaagccagcgtgaccatcgataaatccatcgatgaagtgacgcctgcggagtttgatgccctgctgctaccgggcggccattcaccggattatctgcgtggggacaaccgttttgtcacctttacccgtgattttgtgaatagtggcaaaccggtgtttgccatctgtcacggcccgcagttgctgatcagcgccgatgtgattcgggggcgcaaactgaccgcagttaaaccgatcattattgatgttaaaaatgcgggcgcggaattttacgatcaggaagtcgtggttgataaagatcagctggttaccagccggacaccggacgatctgccagcgtttaaccgcgaggcgttacgcctgctcggtgcc

SEQ ID NO: 5 - protein, 22 aa, synthetic construct
MKYLLPTAAAGLLLLAAQPAMA

SEQ ID NO: 6 - DNA, 66 bp, synthetic construct
  source 1..66: mol_type = other DNA
atgaaatacctgctgccgaccgctgctgctggtctgctgctcctcgctgcccagccggcgatggcc

SEQ ID NO: 7 - protein, 194 aa, synthetic construct
MKYLLPTAAAGLLLLAAQPAMAMSKKIAVLITDEFEDSEFTSPADEFRKAGHEVITIEKQAGKTVKGKKGEASVTIDKSIDEVTPAEFDALLLPGGHSPDYLRGDNRFVTFTRDFVNSGKPVFAICHGPQLLISADVIRGRKLTAVKPIIIDVKNAGAEFYDQEVVVDKDQLVTSRTPDDLPAFNREALRLLGA

SEQ ID NO: 8 - DNA, 585 bp, synthetic construct
  source 1..585: mol_type = other DNA
atgaaatacctgctgccgaccgctgctgctggtctgctgctcctcgctgcccagccggcgatggccatgagtaagaaaattgccgttttaatcactgatgaatttgaggattcagaatttacttcacccgcagacgagttccgtaaagccggacacgaagtgattaccattgaaaaacaagcgggtaaaacggtgaaaggcaaaaaaggagaagccagcgtgaccatcgataaatccatcgatgaagtgacgcctgcggagtttgatgccctgctgctaccgggcggccattcaccggattatctgcgtggggacaaccgttttgtcacctttacccgtgattttgtgaatagtggcaaaccggtgtttgccatctgtcacggcccgcagttgctgatcagcgccgatgtgattcgggggcgcaaactgaccgcagttaaaccgatcattattgatgttaaaaatgcgggcgcggaattttacgatcaggaagtcgtggttgataaagatcagctggttaccagccggacaccggacgatctgccagcgtttaaccgcgaggcgttacgcctgctcggtgcctga